European Patent Specification EP 3 884 951 B1, published October 9, 2024. Title: Composition for Treating Alopecia or Stimulating Hair Growth. Applicant: Medicosbiotech Inc. Korea Advanced Institute of Science and Technology. The sequence listing filed with the application follows.

SEQUENCE LISTING (2 sequences)

SEQ ID NO: 1 - protein, 35 aa, Artificial Sequence
  spider silk peptide
SGRGGLGGQGAGMAAAAAMGGAGQGGYGGLGSQGT

SEQ ID NO: 2 - protein, 38 aa, Artificial Sequence
  sericin silk peptide
SSTGSSSNTDSNSNSVGSSTSGGSSTYGYSSNSRDGSV